European Patent Application EP 4 151 658 A1, published March 22, 2023. Title: SINGLE DOMAIN BINDING MOLECULE. Applicant: Elasmogen Limited. The sequence listing filed with the application follows.

SEQUENCE LISTING (104 sequences)

SEQ ID NO: 1 - protein, 25 aa, Squalus acanthias
TRVDQTPRTATRETGESLTINCVLT

SEQ ID NO: 2 - protein, 10 aa, Squalus acanthias
TYWYRKNPGS

SEQ ID NO: 3 - protein, 8 aa, Squalus acanthias
GRYVESVN

SEQ ID NO: 4 - protein, 20 aa, Squalus acanthias
FSLRIKDLTVADSATYICRA

SEQ ID NO: 5 - protein, 9 aa, Squalus acanthias
GAGTVLTVN

SEQ ID NO: 6 - protein, 8 aa, Squalus acanthias
DTSYPLYS

SEQ ID NO: 7 - protein, 9 aa, Squalus acanthias
MGTNIWTGD

SEQ ID NO: 8 - protein, 9 aa, Squalus acanthias
MATNIWTGD

SEQ ID NO: 9 - protein, 9 aa, Squalus acanthias
MGTDSWTGD

SEQ ID NO: 10 - protein, 9 aa, Squalus acanthias
MGTNSWTGD

SEQ ID NO: 11 - protein, 9 aa, Squalus acanthias
MSTNIWTGD

SEQ ID NO: 12 - protein, 9 aa, Squalus acanthias
ITTDSWTSD

SEQ ID NO: 13 - protein, 9 aa, Squalus acanthias
MGANSWTGD

SEQ ID NO: 14 - protein, 9 aa, Squalus acanthias
MGTNGWTGD

SEQ ID NO: 15 - protein, 9 aa, Squalus acanthias
SDIAMGTYD

SEQ ID NO: 16 - protein, 9 aa, Squalus acanthias
ITTHSWSGD

SEQ ID NO: 17 - protein, 9 aa, Squalus acanthias
LSTYMEAGD

SEQ ID NO: 18 - protein, 9 aa, Squalus acanthias
MDTSAGVVD

SEQ ID NO: 19 - protein, 19 aa, Squalus acanthias
ESPPICTSQGIAAVTKYYD

SEQ ID NO: 20 - protein, 10 aa, Squalus acanthias
  SITE 9: note = X represents Gln
YTIHIKLEXH

SEQ ID NO: 21 - protein, 20 aa, Squalus acanthias
  SITE 18: note = X represents Gln
HAGYGVWNRGLQWRGYDXYD

SEQ ID NO: 22 - protein, 8 aa, Squalus acanthias
YTPGREDY

SEQ ID NO: 23 - protein, 19 aa, Squalus acanthias
EKGRKGSAITSCRRSSYYD

SEQ ID NO: 24 - protein, 13 aa, Squalus acanthias
QSLAISTRSYWYD

SEQ ID NO: 25 - protein, 18 aa, Squalus acanthias
GVAGGYCDYALCSSRYAE

SEQ ID NO: 26 - protein, 9 aa, Squalus acanthias
SNKEQISIS

SEQ ID NO: 27 - protein, 5 aa, Squalus acanthias
KGTKS

SEQ ID NO: 28 - protein, 25 aa, synthetic construct
  REGION 1..25: note = Synthetic sequence: Humanized Framework Region FW1
TRVDQSPSSLSASVGDRVTITCVLT

SEQ ID NO: 29 - protein, 10 aa, synthetic construct
  REGION 1..10: note = Synthetic sequence: Humanized Framework Region FW2
TYWYQQKPGS

SEQ ID NO: 30 - protein, 8 aa, synthetic construct
  REGION 1..8: note = Synthetic sequence: Humanized Framework Region FW3a
GRYSESVN

SEQ ID NO: 31 - protein, 20 aa, synthetic construct
  REGION 1..20: note = Synthetic sequence: Humanized Framework Region FW3b
FTLTISSLQPEDFATYYCRA

SEQ ID NO: 32 - protein, 9 aa, synthetic construct
  REGION 1..9: note = Synthetic sequence: Humanized Framework Region FW4
GAGTKVEIK

SEQ ID NO: 33 - protein, 103 aa, Squalus acanthias
ARVDQTPRTATKETGESLTINCVLTDTSYPLYSTYWYRKNPGSSNKEQISISGRYVESVNKGTKSFSLRIKDLTVADSATYICRAMGTDSWTGDGAGTVLTVN

SEQ ID NO: 34 - protein, 103 aa, Squalus acanthias
IRVDQTPRTATKETGESLTINCVLTDTSYPLYSTYWYRKNPGSSNKEQISISGRYVESVNKGTKSFSLRIKDLTVADSATYICRAMGTNIWTGDGAGTVLTVN

SEQ ID NO: 35 - protein, 103 aa, Squalus acanthias
TRVDQTPRTATKETGESLTINCVLTDTSYPLYSTYWYRKNPGSSNKEQISISGRYVESVNKGTKSFSLRIKDLTVADSATYICRAMGTNSWTGDGAGTALTVN

SEQ ID NO: 36 - protein, 103 aa, Squalus acanthias
ARVDQTPRTATKETGESLTINCVLTDTSYPLYSTYWYRKNPGSSNKEQISISGRYVESVNKGTKSFSLRIKDLTVADSATYICRAMGTNIWTGDGAGTALTVN

SEQ ID NO: 37 - protein, 103 aa, Squalus acanthias
TRVDQTPRTATKETGESLTINCVLTDTSYPLYSTYWYRKNPGSSNKERISISGRYVESVNKGTKSFSLRIKDLTVADSATYICRAMGTBSWTGDGAGTVLTVN

SEQ ID NO: 38 - protein, 103 aa, Squalus acanthias
TRVDQTPRTATKETGESLTINCVLTDTSYPLYRTYWYRKNPGSSNKEQISISGRYVESVNKGTKSFSLRIKDLTVADSATYICRAMGTDSWTGDGAGTVLTVN

SEQ ID NO: 39 - protein, 103 aa, Squalus acanthias
TRVDQTPRTATKETGESLTINCVLTDTSYPLYSTYWYRKNPGSSNKERISISGRYVESVNKGTKSFSLRIKDLTVADSATYICRAMGTDSWTGDGAGTVLTVN

SEQ ID NO: 40 - protein, 103 aa, Squalus acanthias
TRVDQTPRTATKETGESLTINCVLTDTSYPLYSTYWYRKNPGSSNKERISISGRYVESVNKGTKSFSLRIKDLTVADSATYICRAMGTNSWTGDGAGTALTVN

SEQ ID NO: 41 - protein, 103 aa, Squalus acanthias
TRVDQTPRTATKETGESLTINCVLTDTSYPLYSTYWYRKNPGSSNKEQISISGRYVESVNKGTKSFSLRIKDLTVADSATYICRAMGTNIWTGDGAGTALTVN

SEQ ID NO: 42 - protein, 103 aa, Squalus acanthias
TRVDQTPRTATKETGESLTINCVLTDTSYPLYRTYWYRKNPGSSNKEQISISGRYVESVNKGTKSFSLRIKDLTVADSATYICRAMGTNSWTGDGAGTVLTVN

SEQ ID NO: 43 - protein, 103 aa, Squalus acanthias
TRVDQTPRTATKETGESLTINCVLTDTSYPLYSTYWYRKNPGSSNKERISISGRYVESVNKGTKSFSLRIKDLTVADSATYICRAMGTDSWTGDGAGTALTVN

SEQ ID NO: 44 - protein, 103 aa, Squalus acanthias
TRVDQTPRTATKETGESLTINCVLTDTSYPLYSTYWYRKNPGSSNKERISISGRYVESVNKGTKSFSLRIKDLTVADSATYICRAMGTNIWTGDGAGTVLTVN

SEQ ID NO: 45 - protein, 103 aa, Squalus acanthias
TRVDQTPRTATKETGESLTINCVLTDTSYPLYSTYWYRKNPGSSNKEQISISGRYVESVNKGTKSFSLRIKDLTVADSATYICRAMGTNIWTGDGAGTVLTVN

SEQ ID NO: 46 - protein, 103 aa, Squalus acanthias
TRVDQTPRTATRETGESLTINCVLTDTSYPLYSTYWYRKNPGSSNKEQISISGRYVESVNKGTKSFSLRIKDLTVADSATYICRAMGTNIWTGDGAGTVLTVN

SEQ ID NO: 47 - protein, 103 aa, Squalus acanthias
ASVNQTPRTATKETGESLTINCVLTDTSYPLYSTYWYRKNPGSSNKEQISISGRYVESVNKGTKSFSLRIKDLTVADSATYICRAMGTNIWTGDGAGTVLTVN

SEQ ID NO: 48 - protein, 103 aa, Squalus acanthias
ASVNQTPRTATKETGESLTINCVLTDTSYPLYSTYWYRKNPGSSNKEQISISGRYVESVNKGTKSFSLRIKDLTVADSATYICRAMDTSAGVVDGAGTVLTVN

SEQ ID NO: 49 - protein, 103 aa, Squalus acanthias
AKVDQTPRTATKETGESLTINCVLTDTSYPLYSTYWYRKNPGSSNKEQISISGRYVESVNKGTKSFSLRIKDLTVADSATYICRAMGTDSWTGDGAGTVLTVN

SEQ ID NO: 50 - protein, 103 aa, Squalus acanthias
ASVNQTPRTATKETGESLTINCVLTDTSYPLYSTYWYRKNPGSSNKERISISGRYVESVNKGTKSFSLRIKDLTVADSATYICRAMGTDSWTGDGAGTVLTVN

SEQ ID NO: 51 - protein, 112 aa, synthetic construct
  REGION 1..112: note = Synthetic sequence: Specific binding domain E06 with 3xAla -6xHis tag.
TRVDQTPRTATRETGESLTINCVLTDTSYPLYSTYWYRKNPGSSNKEQISISGRYVESVNKGTKSFSLRIKDLTVADSATYICRAMGTNIWTGDGAGTVLTVNAAAHHHHHH

SEQ ID NO: 52 - protein, 113 aa, Squalus acanthias
IRVDQTPRTATKETGESLTINCVLTGTVCGMYSTSWSRKNPGRADWERISIGGRYVESVNKGAKSFSLRIRDLTVADSATYCCSAESPPICTSQGIAAVTKYYDGAGTVLTVN

SEQ ID NO: 53 - protein, 103 aa, Squalus acanthias
ARVDQTPRTATKETGESLTINCVLTDTSYPLYSTYWYRKNPGSSNKEQISISGRYVESVNKGTKSFSLRIKDLTVADSATYICRAITTDSWTSDGAGTALTVN

SEQ ID NO: 54 - protein, 104 aa, Squalus acanthias
  SITE 94: note = X represents Gln
ARVDQTPRTATKETGESLTINCVLTDTSYPLYSTYWYRKNPGSSNKEQISISGRYVESVNKGTKSFSLRIKDLTVADSATYICRAYTIHIKLEXHGAGTVLTVN

SEQ ID NO: 55 - protein, 103 aa, Squalus acanthias
ARVDQTPRTATKETGESLTINCVLTDTSYPLYSTYWYRKNPGSPNKERISISGRYVESVNKGTKSFSLRIKDLTVADSATYICRAMGANSWTGDGAGTALTVN

SEQ ID NO: 56 - protein, 103 aa, Squalus acanthias
ASVNQTPRTATKETGESLTINCVLTDASYPLYSTYWYRKNPGSSNKEQIPISGRYVESVNKGTKSFSLRIKDLTVADSATYICRAMGTNGWTGDGAGTVLTVN

SEQ ID NO: 57 - protein, 114 aa, Squalus acanthias
  SITE 103: note = X represents Gln
AKVDQTPRTTTKETGESLTINCVLTETSYGLSSTSWFQKNPGTTDWERMSIGGRYVESVNTGAKSFSLRIKDLTVADSATYYCKAHAGYGVWNRGLQWRGYDXYDGAGTVLTVN

SEQ ID NO: 58 - protein, 102 aa, Squalus acanthias
TRVDQTPRTATKETGESLTINCVLTDTSYPLYSTYWYRKNPGSSNKEQISISGRYVESVNKGTKSFSLRIKDLTVADSATYICRAYTPGREDYGAGTVLTVN

SEQ ID NO: 59 - protein, 103 aa, Squalus acanthias
ARVDQTPRTATKETGESLTINCVLADTSYPLYSTYWYRKNPGSSNKEQISISGRYVESVNKGTKSFSLRIKDLTVADSATYICRASDIAMGTYDGAGTALTVN

SEQ ID NO: 60 - protein, 113 aa, Squalus acanthias
ASVNQTPRTATKETGESLTINCVLTGTSCSLYSTSWFRKNPGTTDWERISIGGRYVESVNKGAKSFSLRIKDLTVADSATYYCKAEKGRKGSAITSCRRSSYYDGAGTVLTVN

SEQ ID NO: 61 - protein, 103 aa, Squalus acanthias
ARVDQTPRTATKETGESLTINCVLTDTSYPLYSTYWYRKNPGSSNKEQISISGRYVESVNKGTKSFSLRIKDLTVADSGTYICRSITTHSWSGDGAGTALTVN

SEQ ID NO: 62 - protein, 103 aa, Squalus acanthias
IRVDQTPRTATKETGGSLTINCVLTDTSYPLYSTYWYRKNPGSSNKEQISISGRYVESVNKGTKSFSLRIKDLTVADSATYICRALSTYMEAGDGAGTVLTVN

SEQ ID NO: 63 - protein, 103 aa, Squalus acanthias
ASVNQTPRTATKETGESLTINCVLTDTSYPLYSTYWYRKNPGSSNKEQIPISGRYVESVNKGTKSFSLRIKDLTVADSATYICRAMDTSAGVVDGAGTVLTVN

SEQ ID NO: 64 - protein, 107 aa, Squalus acanthias
TRVDQTPRTATKETGESLTINCVLTDTSYGLYSTSWFRKNPGTTDWERMSIGGRYVESVNKGAKSFSLRIKDLTVADSATYYCKAQSLAISTRSYWYDGAGTVLTVN

SEQ ID NO: 65 - protein, 107 aa, Homo sapiens
DIQMTQSPSSLSASVGDRVTITCRASQSISSYLNWYQQKPGKAPKLLIYAASSLQSGVPSRFSGSGSGTDFTLTISSLQPEDFATYYCQQSYSAPRTFGQGTKVEIK

SEQ ID NO: 66 - protein, 113 aa, Ginglymostoma cirratum
ARVDQTPRSVTKETGESLTINCVLRDASYALGSTCWYRKKSGEGNEESISKGGRYVETVNSGSKSFSLRINDLTVEDGGTYRCGLGVAGGYCDYALCSSRYAECGDGTAVTVN

SEQ ID NO: 67 - protein, 112 aa, synthetic construct
  REGION 1..112: note = Synthetic sequence: Humanized shark VNAR 5A7 variant, 5A7 - IVabc
ARVDQSPSSLSASVGDRVTITCVLRDASYALGSTCWYQQKPGKAPKSISKGGRYSESVNSGSKSFTLTISSLQPEDFATYYCGLGVAGGYCDYALCSSRYAECGQGTKVEIK

SEQ ID NO: 68 - protein, 103 aa, synthetic construct
  REGION 1..103: note = Synthetic sequence: Humanized E06 variant
TRVDQSPSSLSASVGDRVTITCVLTDTSYPLYSTYWYQQKPGSSNKEQISISGRYSESVNKGTKSFTLTISSLQPEDFATYYCRAMGTNIWTGDGAGTKVEIK

SEQ ID NO: 69 - protein, 103 aa, synthetic construct
  REGION 1..103: note = Synthetic sequence: Humanized E06 variant
TRVDQSPSSLSASVGDRVTITCVLTDTSYPLYSTYWYQQKPGSSNKEQISISGRYSESVNSGSKSFTLTISSLQPEDFATYYCRAMGTNIWTGDGAGTKVEIK

SEQ ID NO: 70 - protein, 102 aa, synthetic construct
  REGION 1..102: note = Synthetic sequence: Humanized E06 variant
TRVDQSPSSLSASVGDRVTITCVLTDTSYPLYSTYWYQQKPGKAPKQISISGRYSESVNSGSKSFTLTISSLQPEDFATYYCRAMGTNIWTGDGAGTKVEIK

SEQ ID NO: 71 - protein, 103 aa, synthetic construct
  REGION 1..103: note = Synthetic sequence: Humanized E06 variant
DIQMTQSPSSLSASVGDRVTITCVLTDTSYPLYSTYWYQQKPGKAPKQISISGRYSESVNSGSKSFTLTISSLQPEDFATYYCRAMGTNIWTGDGAGTKVEIK

SEQ ID NO: 72 - protein, 101 aa, synthetic construct
  REGION 1..101: note = Synthetic sequence: Humanized E06 variant
TRVDQSPSSLSASVGDRVTITCVLTDTSYPLYSTYWYQQKPGKAPKLQISISGRFSESGSGTDFTLTISSLQPEDFATYYCRAMGTNIWTGDGAGTKVEIK

SEQ ID NO: 73 - protein, 102 aa, synthetic construct
  REGION 1..102: note = Synthetic sequence: Humanized E06 variant
TRVDQSPSSLSASVGDRVTITCVLTDTSYPLYSTYWYQQKPGKAPKQISISGRYSESVNKGTKSFTLTISSLQPEDFATYYCRAMGTNIWTGDGAGTKVEIK

SEQ ID NO: 74 - protein, 103 aa, synthetic construct
  REGION 1..103: note = Synthetic sequence: Humanized E06 variant
TRVDQSPSSLSASVGDRVTITCVLTDTSYPLYSTYWYRKNPGSSNKEQISISGRYSESVNKGTKSFTLTISSLQPEDFATYYCRAMGTNIWTGDGAGTKVEIK

SEQ ID NO: 75 - protein, 103 aa, synthetic construct
  REGION 1..103: note = Synthetic sequence: Humanized E06 variant
ARVDQSPSSLSASVGDRVTITCVLTDTSYPLYSTYWYQQKPGSSNKEQISISGRYSESVNKGTKSFTLTISSLQPEDFATYYCRAMGTNIWTGDGAGTALTVN

SEQ ID NO: 76 - protein, 109 aa, synthetic construct
  REGION 1..109: note = Synthetic sequence: Humanized E06 variant
TRVDQSPSSLSASVGDRVTITCVLTDTSYPLYSTYWYQQKPGKAPKLLIYAASSLQSGVPSRFSGSGSGTDFTLTISSLQPEDFATYYCRAMGTNIWTGDGAGTKVEIK

SEQ ID NO: 77 - protein, 103 aa, synthetic construct
  REGION 1..103: note = Synthetic sequence: Humanized E06 variant
TRVDQSPSSLSASVGDRVTITCVLTDTSYPLYSTYWYRKNPGSSNKEQISISGRYSESVNKGTKSFTLTIKSLQPEDFATYICRAMGTNIWTGDGQGTKVEIK

SEQ ID NO: 78 - protein, 101 aa, synthetic construct
  REGION 1..101: note = Synthetic sequence: Humanized E06 variant
TRVDQSPSSLSASVGDRVTITCVLTDTSYPLYSTYWYRKNPGSSNKEQISISGRYSESGSGTDFTLTIKSLQPEDFATYICRAMGTNIWTGDGQGTKVEIK

SEQ ID NO: 79 - protein, 103 aa, synthetic construct
  REGION 1..103: note = Synthetic sequence: Humanized E06 variant
TRVDQSPSSLSASVGDRVTITCVLTDTSYPLYSTYWYRKNPGSSNKEQISISGRYSESVNKGTKSSTLTISSLQPEDFATYYCRAMGTNIWTGDGAGTKVEIK

SEQ ID NO: 80 - protein, 103 aa, synthetic construct
  REGION 1..103: note = Synthetic sequence: Humanized E06 variant
TRVDQSPSSLSASVGDRVTITCVLTDTSYPLYSTYWYRKNPGSSNKEQISMSGRYSESVNKSTKSFTLTISSLQPEDFATYYCRAMGTNIWTGDGAGTKVEIK

SEQ ID NO: 81 - protein, 103 aa, synthetic construct
  REGION 1..103: note = Synthetic sequence: Humanized E06 variant
TRVDQSPSSLSASVGDRVTITCVLTDTSYPLYSTYWYRKNPGSSNKEQISISGRYSESVNKGTKSFTLTISSLQPEDFATYYCRAMGTNIWTGDGAGTKVETK

SEQ ID NO: 82 - protein, 103 aa, synthetic construct
  REGION 1..103: note = Synthetic sequence: Humanized E06 variant
TRVDQTPSSLSASVGDRVTITCVLTDTSYPLYSTYWYRKNPGSSNKEQISISGRYSESVNKGTKSSTLTISSLQPEDFATYYCRAMGTNIWTGDGAGTKVEIK

SEQ ID NO: 83 - protein, 103 aa, synthetic construct
  REGION 1..103: note = Synthetic sequence: Humanized E06 variant
TRVDQSPSSLSASVGDRVTITCVLTDTSYPLYSTYWYRKNPGSSNKEQISISGRYSESVNKGTKSFTLTISSLQPEDSATYYCRAMSTNIWTGDGAGTKVEIK

SEQ ID NO: 84 - protein, 103 aa, synthetic construct
  REGION 1..103: note = Synthetic sequence: Humanized E06 variant
TRVDQSPSSLSASVGDRVTITCVLTDTSYPLYSTYWYRKNPGSSNKEQISISGRYSESVNKGTKSFTLTISSLQPEDFATYYCRAMGTNFWTGDGAGTKVEIK

SEQ ID NO: 85 - protein, 103 aa, synthetic construct
  REGION 1..103: note = Synthetic sequence: Humanized E06 variant
TRVDQSPSSLSASVGDRVTITCVLTDTSYPLYSTYWYRKNPGSSNKEQISISGRYSESVNKGTKSFTLTISSLQPEDFATYYCRAMATNIWTGDGAGTKVEIK

SEQ ID NO: 86 - protein, 103 aa, synthetic construct
  REGION 1..103: note = Synthetic sequence: Humanized E06 variant
TRVDQSPSSLSASVGDRVTITCVLTDTSYPLYSTYWYRKNPGSNNKEQISISGRYSESVNKGTKSFTLTISSLQPEDFATYYCRAMGTNIWTGDGAGTKVEIK

SEQ ID NO: 87 - protein, 103 aa, synthetic construct
  REGION 1..103: note = Synthetic sequence: Humanized E06 variant
TRVDQSPSSLSASVGDRVTITCVLTDTSYPLYSTYWYRKNPGSSNKEQISISGRYSESVNKGTNSFTLTISSLQPEDFATYYCRAMGTNIWTGDGAGTKVEIK

SEQ ID NO: 88 - protein, 103 aa, synthetic construct
  REGION 1..103: note = Synthetic sequence: Humanized E06 variant
TRVDQSPSSLSASVGDRVTITCVLTDTSYSLYSTYWYRKNPGSSNKEQISISGRYSESVNKGTKSFTLTISSLQPEDFATYYCRAMGTNIWTGDGAGTKVEIK

SEQ ID NO: 89 - protein, 96 aa, synthetic construct
  REGION 1..96: note = Synthetic sequence: Humanized E06 variant
TRVDQSPSSLSASVGDRVTITCVLTDTSYPLYSTYWYRKNPGSSNKEQISISGRYSESVNKGTKSFTLTISSLQPEDFATYYCRAMGTNLWTGDGA

SEQ ID NO: 90 - protein, 9 aa, synthetic construct
  REGION 1..9: note = Synthetic sequence: Peptide linker
AAAHHHHHH

SEQ ID NO: 91 - protein, 8 aa, synthetic construct
  REGION 1..8: note = Synthetic sequence: Humanized Framework Region FW2
TYWYQQKP

SEQ ID NO: 92 - protein, 7 aa, synthetic construct
  REGION 1..7: note = Synthetic sequence: Humanized Framework Region FW3a
RYSESVN

SEQ ID NO: 93 - protein, 18 aa, synthetic construct
  REGION 1..18: note = Synthetic sequence: Humanized Framework Region FW3b
FTLTISSLQPEDFATYYC

SEQ ID NO: 94 - protein, 4 aa, synthetic construct
  REGION 1..4: note = Synthetic sequence: Peptide linker
GGGG

SEQ ID NO: 95 - protein, 5 aa, synthetic construct
  REGION 1..5: note = Synthetic sequence: Peptide linker
GGGGG

SEQ ID NO: 96 - protein, 5 aa, synthetic construct
  REGION 1..5: note = Synthetic sequence: Peptide linker
GGGGS

SEQ ID NO: 97 - protein, 9 aa, synthetic construct
  REGION 1..9: note = Synthetic sequence: Peptide linker
GGGGSGGGG

SEQ ID NO: 98 - protein, 15 aa, synthetic construct
  REGION 1..15: note = Synthetic sequence: Peptide linker
GGGGSGGGGSGGGGS

SEQ ID NO: 99 - protein, 5 aa, Squalus acanthias
SSNKE

SEQ ID NO: 100 - protein, 4 aa, Homo sapiens
KAPK

SEQ ID NO: 101 - protein, 4 aa, Squalus acanthias
TRVD

SEQ ID NO: 102 - protein, 5 aa, Homo sapiens
DIQMT

SEQ ID NO: 103 - protein, 21 aa, Squalus acanthias
  SITE 19: note = X represents Gln
HAGYGVWNRGLQWRGYDDXYD

SEQ ID NO: 104 - protein, 21 aa, Squalus acanthias
HAGYGVWNRGLQWRGYDDYYD